European Patent Specification EP 4 188 910 B1, published July 23, 2025. Title: Compounds with semiochemical properties and biosensors. Applicant: Rothamsted Research Limited. The sequence listing filed with the application follows.

SEQUENCE LISTING (35 sequences)

SEQ ID NO: 1 - protein, 159 aa, Acyrthosiphon pisum
MLNLKVMMFLCLSVIVVYCESDQVPINSSAAVESCLLETNMTRDEFEDMLTSPNARELTILKSHAHKCMFGCVMRKNHIVNDGVVSKEVLSKYVLNFYGRPDYKRRLIIKDVEHIVDVCAKKVADESETDECELAATLVTCIVLEANKAGLVDDPARQI

SEQ ID NO: 2 - protein, 243 aa, Acyrthosiphon pisum
MKVSAATAVLVALVATVQSSDPCNISTCYKSGTTKPPMAVTPTHLPVQSSSTQTSHPQTTYAKDHVHGSTTTKSGVNATVTTASGASVNGTEPPAVVKSSAGVTGNSTTPKPTMTEGHVALKQKLNTIAVKCKDELHAPQEIMALVSNTVVPQNEQQRCYLECVYKNLNLIKNNKFSVEDGKAMARIRFANQPEEHKKAVTIIETCEKEAVIDPKTTEKCAAGRVIRNCFVKNGEKINFFPKA

SEQ ID NO: 3 - protein, 141 aa, Acyrthosiphon pisum
MISSTFYITLVFGIAMLISCGHGRFTTEQIDYYGKACNASEDDLVVVKSYKVPTTETGKCLMKCMITKLGLLNDDGSYNKTGMEAGLKKYWSEWSTEKIESINNKCYEEALLVSKEVVATCNYSYTVMACLNKQLDLDKST

SEQ ID NO: 4 - protein, 193 aa, Acyrthosiphon pisum
MRGNYSSMVFLLFAIGFQDIFCQKQEPSGKCRAPDKAPLNLEIIINTCQEEIKSALLQEALDILNDGNVEQNTPNYSSRSKREAEEDLTNEERRVAGCLLQCVYKKVKAVDETGFPVVDGLMKLYNEGVQDRNYYIATLSAVRHCISIAQQLKQQQPSKSFDDGQTCDLAYEMFECVSEKIEENCGVENKSNN

SEQ ID NO: 5 - protein, 221 aa, Acyrthosiphon pisum
MSANSATIKCIAVAAILLQISVIFADAGHHRRGKELLDTEDSDFFRCKQASRKSCCGPENAMKRFGDKDKVAADECYAQVAEKFATVTATTPKQDLFSAEAVKITKKKQFCLHECIGKKNNLLTEDGSLNKTFIADYAMKSVFKEQWQKQVGQKALDKCLEETYIPWPAEDKENVCNPVYVQFQHCLWLQYESNCPANKIKITKKCEKTRNRYRMQKSTSN

SEQ ID NO: 6 - protein, 215 aa, Acyrthosiphon pisum
MQKVVFICIFAIICQTVFTAGYDRTWILRQKRGTNDDECRTLLPSSEKKLPSCCQMPNILPNLDSTWEKCFETFKQFKDKPETKEYKEMAHGKEPPCLFQCIFMQSGLTTSDGKLNEDAITKKMSEGINNDEKWKSIWQNSLNKCFDDVKQEDKKQILIMNTPAGRLMKCFLRDMYMSCPKNVWVESSECLNMKDLVQKCPEMPPPVFKSPPKLI

SEQ ID NO: 7 - protein, 155 aa, Acyrthosiphon pisum
MVARKRMYNMLPTTVLFAIIAATVLKDCDAYLSEAAIKKTQQMLKTVCSKKHSVEEDVFTNIKKGIFPEDNNNIKCYFACNFKTMQLINQKGVIDKKMFKDKMSMMAPPNVYKILLPVIEQCTGKDKGEELCQSSYNVIKCAHSVDPKSLEFLPL

SEQ ID NO: 8 - protein, 162 aa, Acyrthosiphon pisum
MFALKVACLCLSVAVVFGENNQQNGPSDRSATIFQSCIAETKLSGDALKGFRSMSIPKTQAEKCMMGCLMRKVNVINKGKFSVEEATKVAQKYYGTNEAMMKKAKDLIDVCAKKAQSTTEECALAGIVTTCIVEEAQKAGLSGGPGSRSRRTVSPKFRRDAM

SEQ ID NO: 9 - protein, 165 aa, Acyrthosiphon pisum
MIIKKTLLLSVFVLFGCLFSINKADDADAKDKELMSKLFTVVFKCFKDADWGTCGEMITTKYDITQAKYKQCTCHMACAGEELGMINASGQPEPAKFLEYVNKINNPDIKSQLQLIYDKCQNVKGSEKCDLAEQFAICAFKESPALKERVSTLMEMLVKMKPKSK

SEQ ID NO: 10 - protein, 143 aa, Acyrthosiphon pisum
MEHLRSTNVVFAIVMALLVVQSSTRPQPDEMEEIKRTLYNACAGKFPITEEIKNNAKNSIISDDPTFKCFLKCCFDEMSMIDEDGIIDGDSLKAMAPDHIKPILEQVIPSCTKNVKQDGCEASFEFISCGIKLNPLIVALLPL

SEQ ID NO: 11 - protein, 169 aa, Acyrthosiphon pisum
MSSSTFYITLLFGIAMLISCGYGIFTTEQIDYYGKACNASEDDLIVLKSYKVPSTETGKCLMKCMITKLGLLNDDGSYNKTGMEAGLKKYWSEWATEKIETINEKCYEEGNTATLLYHVAIYFTCVSGDYSDVQLLIHCDGMFEQEVGSRQVNLKLLIMLKIGLSEPKR

SEQ ID NO: 12 - protein, 463 aa, Acyrthosiphon pisum [sequence omitted]

SEQ ID NO: 13 - protein, 403 aa, Acyrthosiphon pisum
MDVMQKPERFILTPFQKFCIRWSVFFDSSSDRLSRIETVLRTIQFSTIMITSGMTMTSVLIADNKKALESFTYFVICVFMLAIITFAIRTKRFNRAMLLMVVDEFPGYNRPMPDVLKRKMAAIRTSYGDFTMKVIVSYLTLVLFEIPATAMVPLAAASLTDVKLGSQSTQMVVLWFPADTSQVGMYAVSYVIQFLIVVTVKFIITGIMCSFSFFVSQMISEFQILSAYVEHAVEIVEYDQSADKTTEQKLLDHVKNCVMLHDRLIYFKDQLNESYGYIILLELMFSTLYFCLSAFNMIFVGNRFVMVKGLLTLSNYLAELFIFCMYGSMVEDAHMGLLRASYSVAWYAQPVRFRQSLTMVMSRTQTPLQLTVGKVFIANLPLFLSVLKVSYSGVNALRAANAK

SEQ ID NO: 14 - protein, 386 aa, Acyrthosiphon pisum
MTSIGKKNQRKFYQTLMTLAFFLDTSQYRYISRFVKQFYIFDWMVLVSVAAAFTILEGNYRMPFVMELIQYMIVGFYFTSIFVVFIIKKEAIMSNYNCIQTKFIQWSNKRALHSNAAYKRNIKTVKSLSIPLAILSLSIALGPLISTINDIGKLPLDNRAHFVLFWPTIVDTNKLSMYGIIYTLQVIFTIILYISVLSFNLGYMVFLNELITQFEMLLNGINDAFKYKMDKQFQTLFIDCIRHHQIIIKFLDDLKSYFKWMILIEIIVVQVILAILIYNLTKVNASLGYKVKIAGSILFNLLPICFHCHVGEVVLSLHTRLSNHIYNMPWYDMPNKNKQLIVIMLQRTQRDLTLSSALFSSERASRSLISKVIKQVYTILNVLLKT

SEQ ID NO: 15 - protein, 367 aa, Acyrthosiphon pisum
MQRIDTINMFLQMTGCTDSKAMLYLTYFEFLITFYYLIATYASIVHFEQSVTIQLFALLCMLIECVILLNITFRLYHKNHIREMHQYSRRLGIPDSYRSVINVITKYHLIASNIFVVFPVTYAIFCDSVRVGDPFTFPFLDVLPMHTDNLAIYACKYLVYAISVYIAHVELCFINTTFIYYVGVLKHRLETIVQTIGEAFADNDEQKFKYAIIQHQKLLSYFNTMKIVFSKPILLSMSFNAIYFGLTTSFVIQAIRGYINQAILSICIASSAAAVINITIYTFYGSELMDLHDKILHVLFDNAFFYVSKSFKSSILIMMTRVTIPLKFTVGYIFTINLNLLLKILKMSYTVLNVLLSSETIKPHKLS

SEQ ID NO: 16 - protein, 369 aa, Acyrthosiphon pisum
MAHIVDIFFQNMGCSHDHGYGMVFFNCCELAITLFFTVSTYPTIADPTQNLSIRLYGVLCLLIEAHIFAFIAVRIYHQSQHRDMYQHLHGVEIPENYRRKIATVIKHHFIISNVFVAVSVLYTISLDWVRIGDPFTFPFIDVLPIKTTNVTVYVCKYIVYALPVYFAHLETCFLNVTFMFSVGIVKRHFQILNDQVEEAIVNEDEQKLKIAIKHHQQVLKYFEDMKTVYEKPILMTIEFCGLYVGLTSCFVIQVIQGFIHQIILGLCIVSSIACLMTIIIYCIYASNMYALHNGILNALFEHRSCYSRNKSFKRIILIMMTRATIPLEIKAGSVFTINLNLLVKILKFAYTVFNVLLSSINRQFKETAI

SEQ ID NO: 17 - protein, 430 aa, Acyrthosiphon pisum
MTTTPRVTELTAPASEDLTIVDNRLFKAICLHQILDPTKGGNRYYRLAFMVVMWVSLSVQIIQLVGLYFAVNDLQRFAFTTTVIFNALLCLSKGYVLVVNADRLRASLEVARYEFTSCGARNQRLVRRSRAVLSTILRTFAVLSWVTCFIWALTPLFAMDEYLQVTNADGTVSRYRVTIYNVWLPVPATVYNETTVWSLVYAVEVIACFVNVFSWLLFDSYVVTMCFTFNAQFRTVSASTTIGHHSDSFRSPPPHAPEGTSDDNNTFNCYDELINRIKDNQSIIKIYDDFFEILQPAILFQIIGGSYSVITLIFLTSLTYLMGFSIISIPVLKVFFGFLSVTFELFLYCYVFNHIETEKCNMNFGLYSSNWTAMDLKFKKTLLFAMNTNSSHRRVMKVTPMSIINLEMFANVMNMSYSIVSVLLNSRVQK

SEQ ID NO: 18 - protein, 420 aa, Acyrthosiphon pisum
MRSSSATVVDVMLFKAIGLYQLLCPADRGGYSVRSRRALMTALGLSFALHSFQVPYLYYALNDLQRFAYMAAVIIYGMMCSFKGYVLVTNADRLWLVLNAADYGYTGCGHRDPSRLRRCRATLSALLRTFVALSYGTLIVWIVLPFFVDEYTGITNSDGTVTRYRTTIHNMQYPIPLAVYNSRPVWALIYVTELYVCIVNVFIWSLFDCYLVTMCFVLNAQFHTMSAGYGTLGIRRTGSSPPDTTFAGVRRIKFDEIESNHYSDLISHIQDNQNLIKMFDVFFEVVRPVVLVQIANGSYSVISLIFLTALMYLMGVPVLSAAFLKFICGLISLTIELFIFCYGFNHIETAKSVLNFGIYSSNWTEMDLTFKKTMLLTMKMNSSHKRAMKVSPNSAVGLEMFARVMNMSYSTVSVLLNSRS

SEQ ID NO: 19 - protein, 388 aa, Acyrthosiphon pisum
FKHQGLVADLLPNIRVMQGVGHFMFNYYSEGKKFPHRIYCIVTLLLLLLQYGMMAVNLMMESDDVDDLTANTITMLFFLHPIVKMIYFPVRSKIFYKTLAIWNNPNSHPLFAESNARFHALAITKMRRLLFCVAGATIFSVISWTGITFIEDSPIPRLMIRTFYPFNAMSGAGHVFALIYQFYYLVISMAVSNSLDVLFCSWLLFACEQLQHLKAIMKPLMELSATGLTKKQEMLVRSAIKYWVERHKHVVRLVTAVGDAYGVALLLHMLTTTITLTLLAYQATKVNGVNVYAATVIGYLLYTLGQVFLFCIFGNRLIEESSSVMEAAYSCHWYDGSEEAKTFVQIVCQQCQKAMSISGAKFFTVSLDLFASVLGAVVTYFMVLVQLK

SEQ ID NO: 20 - protein, 414 aa, Acyrthosiphon pisum
MNLNDEQNYIVNLKLMKITGFYHLISSRAPKYFGFNVYKVTAAIEVMTGIFSIIMLFLSSYYYLDNTNELMSHFMLVVAIFFSTLKIFWVSRNSETIWNNMDMTCINFLSYTGHKKEILKKARAKSISTTILFVILWSSVTVAWSISPFFVKDVYLNIKFKDETRRFRYNSLNYVYPISEEFYNEHFLYFYVVEMLSVVFWGHGTVAYDTFVISICITIAFQLKTIAVSYISLNDKKGDIKNLKDNDLEAMFNLKLLIQDQQNMFKKIKEIYKIFEPVTFVQLAAQSMLIILQAYMIFINHYNGFSLLSVPIIKLIVTVAPNIIHLFITCYLYTNINHQQDSMNFALYSSDWTAMSINYKKMLLFTMRMNDAEKLKLKISLRKIVNLEMFASVMHLTYSIISVLAKSYGNTNTK

SEQ ID NO: 21 - protein, 424 aa, Acyrthosiphon pisum
MATGIKTVSKNEDNFMINMRLMKKTGFYQLLDSRSLKVFGHNVFKCMSVVQMSILSSVAFIFVANIYYFSDDINTVMMYSMLITSDVLSILKLYYILQNSDTIWNCIQMTSIDDLSYKYHDRRILEEGRSKSTSYSILIMFMWLNLIVSWSLGPLFVTNYFLIVEQNDEIYRYRFNIMNFAFPATDRFYNDNFMIYYGIEFITLVLWCHCTMNFDVLLLSMNITFKYQLKTISNSFSAFNFTRYNDFKNNRTKNVKHHKESESMFDFKSLIYDQQRVIENMKNIYRVFRPVVLTQLASESLIIMLLSCIIMLNYFNGISLLSALNLRIFAAISTFLFHIYVICYLFDDVNEQKDSMNLALYSSDWTTSDLQHKILLLHAMRMNNAENLRLQVTRNKIVNFQMFTYVRMIFFSFYYSGYCGHYFY

SEQ ID NO: 22 - protein, 437 aa, Acyrthosiphon pisum
MNPTFKHFFKGDCTNITKPSPMETCIDHTCTINLNILKQCGFYQIFDPNSKKIFGWNVYRISFIALTVITQCLIGFGNCGFLFELEDTTDNIDLFLIIFSNSYFCLTEWKVVILIINRKKFLELLDVTDLIFLKSKQCRKNIKILCKHRIRALQLTNLYFKFCIFVIIEWIIFPIMINSFIAHKTENRRLENVVNRRYPVDVNTYNKYYILFYVFEIIIGVKTVYLVLMVDILLLSIGWAIVIQYEVLAEAFKNIGYNENLQKDHDHDVDDYKYFKSILFDQQQLDSKVKLYFPIVKPIVLMHVAINSVLFIMLSNSFLMVFLSTESFTYKIVNLFKIGTGILYICLQLFLYCHLFDNINLKRKSVNLGIYSCNWTKMDLKFKKLLLLTMQINDANYITIKASTKTIVNLPIFANVLMTSYNIVSVMVKTMSKYRKT

SEQ ID NO: 23 - protein, 416 aa, Acyrthosiphon pisum
MKWLQDHEVAINLALFKRYQFYQIFNPNGSKLLNYDTYKLTNVMFIVAVTTYNIFSAMCFFTDTIDTIDSVDLLLMIFIYSIIIISLLKISVLLFNADQIWELFDLTRFDFLTSRQCRKNVGILCKYRDRSITITNLYQNYSTMVFIIWMITPLVLNTFVVVGGPNQRYHNIFNMQYPVSANIYNQYYYLFYLMEIAMGIFVLNYSMIVDNFLISLCWVIIAQYEVITTAFEKIGNDCELTTLQNEKNNNSFEAYEDLKSILMDQNKLYIKLKSFYRVVWIIVIFLIIIDSVLLIILTYSFVMICSSAESFSIFNILKISTAFFVFVIQLYLYCYLFDVLNDKKESVNFGLYCCDWTKMDLRFKKLLLLATKFNNANTLKIKSTPNKIVNLQLFSSVMTTAFNIVTVMLKTMNGKN

SEQ ID NO: 24 - protein, 424 aa, Acyrthosiphon pisum
MGIDNMSSLKSNEVAINLKLFKVFRFYHIFDPNSGKLCKFNVYHLAWYIINCVIGCILIYGLLGYFTEMEDVIDSIFHIQIMFCYLLYSLSLLKIITFLYKANNIWDLLRVTRINFLTSTQCQAHIGILHKHRNKSIKITNLISGFAIVTTLEWILFPLVLRLLSKTDASHSNKRFENIFNFRFPVTVCEYNNYYFIFYIMESFIAIFMLYAYVVTDVFFISVCYVIIAQYEIIKRAYEIVNCEQTSENNNENKNHNNIIVNDCCDDLISIVMDQQNHYAKLRLFYSTYKLIIVSTVVINSGSIIILTYASVVIFTSPETIPILSIVKLISAFTYMFFVLFFLCYLMECINNKIESVQLGMYSCNWTAMNIKSKKLLLFSMRMHNANKLMIKTTPNNIINLQLFNSVMMTSYNIVSAMVNTRSK

SEQ ID NO: 25 - protein, 426 aa, Acyrthosiphon pisum
MFSCDFINRTVNMNSENLFNGGSVAFNLSTYKQLGYYQLLDPKGPHIYGYHLYRTILKIFLLIVQFITIFGVMGFFIEMEDTDPGKSNSFELIIILTNCSLSSLKIYTLISNSKIIWDLFDLTRIDFLRCSRHSKLITKNFVKRCKKSTTITKWIARSFLVGLILWLMGPFIANEEHTEPNTVHRHKNIINIKFPVTMKTYNNYYFVFYLMEVAVGFCIVYGSVLIDAYLMSFCWIISAQYQSVTKAFATFGYNKQGSPKDIYKDFKSIIIDHQNIYLKMKSFYAVVRPITLIHVFAYSCSLIMYAYVIVTIFNSKELFIIAEIMKIVMTVSNVTMEVFIFCYLFELIDNKKEDVNFGLYSCNWTGMDIKFKQLLLMSMKMNNANRFKLKASPDVTINRPFFANVIHTCFKIVSVLIQTQSIDLLN

SEQ ID NO: 26 - protein, 427 aa, Acyrthosiphon pisum
MPNSSEECVMSSSMAKCTGLHYIIDPEGPTVGGHNVFHVTVMVMIGFTVVCLSMCPFGLYYWANDVTQCIFLLIYIVNFSFGCFKAFTLVRHSDDICRCLDVTRFDFSSGAIMSDPDSARFFRKCRDASSTFTGWFAASSHFVLLVWTLLPFVVVGKGVEINNRDGSTSYYHFNPYNMYFLVSSETYNRLHLVFHLVEWAFGLCFVLIMVAFDTFMVTLCVAITCQMRGIGNAYSKLGHDRCATASNVCSDGGIESNKSNNEYLRDLKLIIKDHQAVLGKMNDFYKIVGPVILPQLIVASFTIIFVSFIITRNYFNGMLLTSTQSLKMCCFPIFFYQVYYTCHAFGNLSHRKNVMNFALYSSDWTQMEIKFKKLLLLAMQMHDANKLDMKLTDKLVINLELFTRVINMCYSIFSVLVNSQLKIADKQ

SEQ ID NO: 27 - protein, 422 aa, Acyrthosiphon pisum
MDSKQEKQYIFNMKLARIMGLYQILFPNSTSFFGYNIYHVVTVFFVSFTFAISMLFPIGLLYLRNDIIAIMYYMGCISNFLLSCFKMVNILYHSKDIWKCIDVTSFNYILYKHYDRNVFKNWQTRSIRITYIYIVIALFAFFCWIFSPCIMNKSVIAIRNIDGSYSKYRMNIFNLYLIASNETYNKNFYIFYVIEIIISICYVYFTIVFDVLMLLVCFAISYQLETISNTIKSLGHEIYTRDNIRSGNSIKLKEKHGILYNDLITIMTDHQNVLKKLNDFYNIFRSITLTQIFIASSSHVFIWFIAAMSIDEGDNADSILSFKLFIVLPLINFQLFMTCSLFGTINEKKDSIIFALYSSNWTNMDLKSKKMILFNLTINNASQLKMKFTNTKIVNLEMFSHTMRFCYSIFSMLINYNKNKMK

SEQ ID NO: 28 - DNA, 29 bp, Artificial Sequence
  Synthetic - forward primer
cgcggcagcgctgggtacgatagaacatg

SEQ ID NO: 29 - DNA, 27 bp, Artificial Sequence
  Synthetic - reverse primer
cggcaccagcggatccggactcttgtc

SEQ ID NO: 30 - protein, 23 aa, Artificial Sequence
  Synthetic - pET45b His-Tag FASTA sequence
MAHHHHHHVGTGSNDDDDKSPDP

SEQ ID NO: 31 - protein, 22 aa, Artificial Sequence
  Synthetic - pNIC28-Bsa4 His-Tag FASTA sequence
MHHHHHHSSGVDLGTENLYFQS

SEQ ID NO: 32 - protein, 20 aa, Artificial Sequence
  Synthetic - pET15b His-Tag FASTA sequence
MGSSHHHHHHSSGLVPRGSH

SEQ ID NO: 33 - protein, 6 aa, Artificial Sequence
  Synthetic - pET45b cleavage site
DDDDKS

SEQ ID NO: 34 - protein, 7 aa, Artificial Sequence
  Synthetic - pNIC28-Bsa4 cleavage site
ENLYFQS

SEQ ID NO: 35 - protein, 7 aa, Artificial Sequence
  Synthetic - pET15b cleavage site
GLVPRGS